European Patent Application EP 4 130 047 A1, published February 8, 2023. Title: 可溶性ACE2和融合蛋白，及其应用. Applicant: 华辉安健（北京）生物科技有限公司. The sequence listing filed with the application follows.

SEQUENCE LISTING (18 sequences)

SEQ ID NO: 1 - protein, 596 aa, Homo sapiens
TIEEQAKTFLDKFNHEAEDLFYQSSLASWNYNTNITEENVQNMNNAGDKWSAFLKEQSTLAQMYPLQEIQNLTVKLQLQALQQNGSSVLSEDKSKRLNTILNTMSTIYSTGKVCNPDNPQECLLLEPGLNEIMANSLDYNERLWAWESWRSEVGKQLRPLYEEYVVLKNEMARANHYEDYGDYWRGDYEVNGVDGYDYSRGQLIEDVEHTFEEIKPLYEHLHAYVRAKLMNAYPSYISPIGCLPAHLLGDMWGRFWTNLYSLTVPFGQKPNIDVTDAMVDQAWDAQRIFKEAEKFFVSVGLPNMTQGFWENSMLTDPGNVQKAVCHPTAWDLGKGDFRILMCTKVTMDDFLTAHHEMGHIQYDMAYAAQPFLLRNGANEGFHEAVGEIMSLSAATPKHLKSIGLLSPDFQEDNETEINFLLKQALTIVGTLPFTYMLEKWRWMVFKGEIPKDQWMKKWWEMKREIVGVVEPVPHDETYCDPASLFHVSNDYSFIRYYTRTLYQFQFQEALCQAAKHEGPLHKCDISNSTEAGQKLFNMLRLGKSEPWTLALENVVGAKNMNVRPLLNYFEPLFTWLKDQNKNSFVGWSTDWSPYAD

SEQ ID NO: 2 - protein, 596 aa, Artificial Sequence
  Artificial Sequence
TIEEQAKTFLDKFNHEAEDLFYQSSLASWNYNTNITEENVQNMNNAGDKWSAFLKEQSTLAQMYPLQEIQNLTVKLQLQALQQNGSSVLSEDKSKRLNTILNTMSTIYSTGKVCNPDNPQECLLLEPGLNEIMANSLDYNERLWAWESWRSEVGKQLRPLYEEYVVLKNEMARANHYEDYGDYWRGDYEVNGVDGYDYSRGQLIEDVEHTFEEIKPLYEHLHAYVRAKLMNAYPSYISPIGCLPAHLLGDMWGRFWTNLYSLTVPFGQKPNIDVTDAMVDQAWDAQRIFKEAEKFFVSVGLPNMTQGFWENSMLTDPGNVQKAVCHPTAWDLGKGDFRILMCTKVTMDDFLTAHNEMGNIQYDMAYAAQPFLLRNGANEGFHEAVGEIMSLSAATPKHLKSIGLLSPDFQEDNETEINFLLKQALTIVGTLPFTYMLEKWRWMVFKGEIPKDQWMKKWWEMKREIVGVVEPVPHDETYCDPASLFHVSNDYSFIRYYTRTLYQFQFQEALCQAAKHEGPLHKCDISNSTEAGQKLFNMLRLGKSEPWTLALENVVGAKNMNVRPLLNYFEPLFTWLKDQNKNSFVGWSTDWSPYAD

SEQ ID NO: 3 - protein, 828 aa, Artificial Sequence
  Artificial Sequence
TIEEQAKTFLDKFNHEAEDLFYQSSLASWNYNTNITEENVQNMNNAGDKWSAFLKEQSTLAQMYPLQEIQNLTVKLQLQALQQNGSSVLSEDKSKRLNTILNTMSTIYSTGKVCNPDNPQECLLLEPGLNEIMANSLDYNERLWAWESWRSEVGKQLRPLYEEYVVLKNEMARANHYEDYGDYWRGDYEVNGVDGYDYSRGQLIEDVEHTFEEIKPLYEHLHAYVRAKLMNAYPSYISPIGCLPAHLLGDMWGRFWTNLYSLTVPFGQKPNIDVTDAMVDQAWDAQRIFKEAEKFFVSVGLPNMTQGFWENSMLTDPGNVQKAVCHPTAWDLGKGDFRILMCTKVTMDDFLTAHHEMGHIQYDMAYAAQPFLLRNGANEGFHEAVGEIMSLSAATPKHLKSIGLLSPDFQEDNETEINFLLKQALTIVGTLPFTYMLEKWRWMVFKGEIPKDQWMKKWWEMKREIVGVVEPVPHDETYCDPASLFHVSNDYSFIRYYTRTLYQFQFQEALCQAAKHEGPLHKCDISNSTEAGQKLFNMLRLGKSEPWTLALENVVGAKNMNVRPLLNYFEPLFTWLKDQNKNSFVGWSTDWSPYADEPKSSDKTHTCPPCPAPELLGGPSVFLFPPKPKDTLMISRTPEVTCVVVDVSHEDPEVKFNWYVDGVEVHNAKTKPREEQYNSTYRVVSVLTVLHQDWLNGKEYKCKVSNKALPAPIEKTISKAKGQPREPQVYTLPPSRDELTKNQVSLTCLVKGFYPSDIAVEWESNGQPENNYKTTPPVLDSDGSFFLYSKLTVDKSRWQQGNVFSCSVMHEALHNHYTQKSLSLSPGK

SEQ ID NO: 4 - protein, 828 aa, Artificial Sequence
  Artificial Sequence
TIEEQAKTFLDKFNHEAEDLFYQSSLASWNYNTNITEENVQNMNNAGDKWSAFLKEQSTLAQMYPLQEIQNLTVKLQLQALQQNGSSVLSEDKSKRLNTILNTMSTIYSTGKVCNPDNPQECLLLEPGLNEIMANSLDYNERLWAWESWRSEVGKQLRPLYEEYVVLKNEMARANHYEDYGDYWRGDYEVNGVDGYDYSRGQLIEDVEHTFEEIKPLYEHLHAYVRAKLMNAYPSYISPIGCLPAHLLGDMWGRFWTNLYSLTVPFGQKPNIDVTDAMVDQAWDAQRIFKEAEKFFVSVGLPNMTQGFWENSMLTDPGNVQKAVCHPTAWDLGKGDFRILMCTKVTMDDFLTAHNEMGNIQYDMAYAAQPFLLRNGANEGFHEAVGEIMSLSAATPKHLKSIGLLSPDFQEDNETEINFLLKQALTIVGTLPFTYMLEKWRWMVFKGEIPKDQWMKKWWEMKREIVGVVEPVPHDETYCDPASLFHVSNDYSFIRYYTRTLYQFQFQEALCQAAKHEGPLHKCDISNSTEAGQKLFNMLRLGKSEPWTLALENVVGAKNMNVRPLLNYFEPLFTWLKDQNKNSFVGWSTDWSPYADEPKSSDKTHTCPPCPAPELLGGPSVFLFPPKPKDTLMISRTPEVTCVVVDVSHEDPEVKFNWYVDGVEVHNAKTKPREEQYNSTYRVVSVLTVLHQDWLNGKEYKCKVSNKALPAPIEKTISKAKGQPREPQVYTLPPSRDELTKNQVSLTCLVKGFYPSDIAVEWESNGQPENNYKTTPPVLDSDGSFFLYSKLTVDKSRWQQGNVFSCSVMHEALHNHYTQKSLSLSPGK

SEQ ID NO: 5 - protein, 844 aa, Artificial Sequence
  Artificial Sequence
MPLLLLLPLLWAGALATIEEQAKTFLDKFNHEAEDLFYQSSLASWNYNTNITEENVQNMNNAGDKWSAFLKEQSTLAQMYPLQEIQNLTVKLQLQALQQNGSSVLSEDKSKRLNTILNTMSTIYSTGKVCNPDNPQECLLLEPGLNEIMANSLDYNERLWAWESWRSEVGKQLRPLYEEYVVLKNEMARANHYEDYGDYWRGDYEVNGVDGYDYSRGQLIEDVEHTFEEIKPLYEHLHAYVRAKLMNAYPSYISPIGCLPAHLLGDMWGRFWTNLYSLTVPFGQKPNIDVTDAMVDQAWDAQRIFKEAEKFFVSVGLPNMTQGFWENSMLTDPGNVQKAVCHPTAWDLGKGDFRILMCTKVTMDDFLTAHHEMGHIQYDMAYAAQPFLLRNGANEGFHEAVGEIMSLSAATPKHLKSIGLLSPDFQEDNETEINFLLKQALTIVGTLPFTYMLEKWRWMVFKGEIPKDQWMKKWWEMKREIVGVVEPVPHDETYCDPASLFHVSNDYSFIRYYTRTLYQFQFQEALCQAAKHEGPLHKCDISNSTEAGQKLFNMLRLGKSEPWTLALENVVGAKNMNVRPLLNYFEPLFTWLKDQNKNSFVGWSTDWSPYADEPKSSDKTHTCPPCPAPELLGGPSVFLFPPKPKDTLMISRTPEVTCVVVDVSHEDPEVKFNWYVDGVEVHNAKTKPREEQYNSTYRVVSVLTVLHQDWLNGKEYKCKVSNKALPAPIEKTISKAKGQPREPQVYTLPPSRDELTKNQVSLTCLVKGFYPSDIAVEWESNGQPENNYKTTPPVLDSDGSFFLYSKLTVDKSRWQQGNVFSCSVMHEALHNHYTQKSLSLSPGK

SEQ ID NO: 6 - protein, 844 aa, Artificial Sequence
  Artificial Sequence
MPLLLLLPLLWAGALATIEEQAKTFLDKFNHEAEDLFYQSSLASWNYNTNITEENVQNMNNAGDKWSAFLKEQSTLAQMYPLQEIQNLTVKLQLQALQQNGSSVLSEDKSKRLNTILNTMSTIYSTGKVCNPDNPQECLLLEPGLNEIMANSLDYNERLWAWESWRSEVGKQLRPLYEEYVVLKNEMARANHYEDYGDYWRGDYEVNGVDGYDYSRGQLIEDVEHTFEEIKPLYEHLHAYVRAKLMNAYPSYISPIGCLPAHLLGDMWGRFWTNLYSLTVPFGQKPNIDVTDAMVDQAWDAQRIFKEAEKFFVSVGLPNMTQGFWENSMLTDPGNVQKAVCHPTAWDLGKGDFRILMCTKVTMDDFLTAHNEMGNIQYDMAYAAQPFLLRNGANEGFHEAVGEIMSLSAATPKHLKSIGLLSPDFQEDNETEINFLLKQALTIVGTLPFTYMLEKWRWMVFKGEIPKDQWMKKWWEMKREIVGVVEPVPHDETYCDPASLFHVSNDYSFIRYYTRTLYQFQFQEALCQAAKHEGPLHKCDISNSTEAGQKLFNMLRLGKSEPWTLALENVVGAKNMNVRPLLNYFEPLFTWLKDQNKNSFVGWSTDWSPYADEPKSSDKTHTCPPCPAPELLGGPSVFLFPPKPKDTLMISRTPEVTCVVVDVSHEDPEVKFNWYVDGVEVHNAKTKPREEQYNSTYRVVSVLTVLHQDWLNGKEYKCKVSNKALPAPIEKTISKAKGQPREPQVYTLPPSRDELTKNQVSLTCLVKGFYPSDIAVEWESNGQPENNYKTTPPVLDSDGSFFLYSKLTVDKSRWQQGNVFSCSVMHEALHNHYTQKSLSLSPGK

SEQ ID NO: 7 - protein, 862 aa, Artificial Sequence
  Artificial Sequence
MPLLLLLPLLWAGALATIEEQAKTFLDKFNHEAEDLFYQSSLASWNYNTNITEENVQNMNNAGDKWSAFLKEQSTLAQMYPLQEIQNLTVKLQLQALQQNGSSVLSEDKSKRLNTILNTMSTIYSTGKVCNPDNPQECLLLEPGLNEIMANSLDYNERLWAWESWRSEVGKQLRPLYEEYVVLKNEMARANHYEDYGDYWRGDYEVNGVDGYDYSRGQLIEDVEHTFEEIKPLYEHLHAYVRAKLMNAYPSYISPIGCLPAHLLGDMWGRFWTNLYSLTVPFGQKPNIDVTDAMVDQAWDAQRIFKEAEKFFVSVGLPNMTQGFWENSMLTDPGNVQKAVCHPTAWDLGKGDFRILMCTKVTMDDFLTAHHEMGHIQYDMAYAAQPFLLRNGANEGFHEAVGEIMSLSAATPKHLKSIGLLSPDFQEDNETEINFLLKQALTIVGTLPFTYMLEKWRWMVFKGEIPKDQWMKKWWEMKREIVGVVEPVPHDETYCDPASLFHVSNDYSFIRYYTRTLYQFQFQEALCQAAKHEGPLHKCDISNSTEAGQKLFNMLRLGKSEPWTLALENVVGAKNMNVRPLLNYFEPLFTWLKDQNKNSFVGWSTDWSPYADEPKSSDKTHTCPPCPAPELLGGPSVFLFPPKPKDTLMISRTPEVTCVVVDVSHEDPEVKFNWYVDGVEVHNAKTKPREEQYNSTYRVVSVLTVLHQDWLNGKEYKCKVSNKALPAPIEKTISKAKGQPREPQVYTLPPSRDELTKNQVSLTCLVKGFYPSDIAVEWESNGQPENNYKTTPPVLDSDGSFFLYSKLTVDKSRWQQGNVFSCSVMHEALHNHYTQKSLSLSTGKPTLYNVSLVMSDTAGTCY

SEQ ID NO: 8 - protein, 862 aa, Artificial Sequence
  Artificial Sequence
MPLLLLLPLLWAGALATIEEQAKTFLDKFNHEAEDLFYQSSLASWNYNTNITEENVQNMNNAGDKWSAFLKEQSTLAQMYPLQEIQNLTVKLQLQALQQNGSSVLSEDKSKRLNTILNTMSTIYSTGKVCNPDNPQECLLLEPGLNEIMANSLDYNERLWAWESWRSEVGKQLRPLYEEYVVLKNEMARANHYEDYGDYWRGDYEVNGVDGYDYSRGQLIEDVEHTFEEIKPLYEHLHAYVRAKLMNAYPSYISPIGCLPAHLLGDMWGRFWTNLYSLTVPFGQKPNIDVTDAMVDQAWDAQRIFKEAEKFFVSVGLPNMTQGFWENSMLTDPGNVQKAVCHPTAWDLGKGDFRILMCTKVTMDDFLTAHNEMGNIQYDMAYAAQPFLLRNGANEGFHEAVGEIMSLSAATPKHLKSIGLLSPDFQEDNETEINFLLKQALTIVGTLPFTYMLEKWRWMVFKGEIPKDQWMKKWWEMKREIVGVVEPVPHDETYCDPASLFHVSNDYSFIRYYTRTLYQFQFQEALCQAAKHEGPLHKCDISNSTEAGQKLFNMLRLGKSEPWTLALENVVGAKNMNVRPLLNYFEPLFTWLKDQNKNSFVGWSTDWSPYADEPKSSDKTHTCPPCPAPELLGGPSVFLFPPKPKDTLMISRTPEVTCVVVDVSHEDPEVKFNWYVDGVEVHNAKTKPREEQYNSTYRVVSVLTVLHQDWLNGKEYKCKVSNKALPAPIEKTISKAKGQPREPQVYTLPPSRDELTKNQVSLTCLVKGFYPSDIAVEWESNGQPENNYKTTPPVLDSDGSFFLYSKLTVDKSRWQQGNVFSCSVMHEALHNHYTQKSLSLSTGKPTLYNVSLVMSDTAGTCY

SEQ ID NO: 9 - protein, 1273 aa, Coaxana purpurea
MFVFLVLLPLVSSQCVNLTTRTQLPPAYTNSFTRGVYYPDKVFRSSVLHSTQDLFLPFFSNVTWFHAIHVSGTNGTKRFDNPVLPFNDGVYFASTEKSNIIRGWIFGTTLDSKTQSLLIVNNATNVVIKVCEFQFCNDPFLGVYYHKNNKSWMESEFRVYSSANNCTFEYVSQPFLMDLEGKQGNFKNLREFVFKNIDGYFKIYSKHTPINLVRDLPQGFSALEPLVDLPIGINITRFQTLLALHRSYLTPGDSSSGWTAGAAAYYVGYLQPRTFLLKYNENGTITDAVDCALDPLSETKCTLKSFTVEKGIYQTSNFRVQPTESIVRFPNITNLCPFGEVFNATRFASVYAWNRKRISNCVADYSVLYNSASFSTFKCYGVSPTKLNDLCFTNVYADSFVIRGDEVRQIAPGQTGKIADYNYKLPDDFTGCVIAWNSNNLDSKVGGNYNYLYRLFRKSNLKPFERDISTEIYQAGSTPCNGVEGFNCYFPLQSYGFQPTNGVGYQPYRVVVLSFELLHAPATVCGPKKSTNLVKNKCVNFNFNGLTGTGVLTESNKKFLPFQQFGRDIADTTDAVRDPQTLEILDITPCSFGGVSVITPGTNTSNQVAVLYQDVNCTEVPVAIHADQLTPTWRVYSTGSNVFQTRAGCLIGAEHVNNSYECDIPIGAGICASYQTQTNSPRRARSVASQSIIAYTMSLGAENSVAYSNNSIAIPTNFTISVTTEILPVSMTKTSVDCTMYICGDSTECSNLLLQYGSFCTQLNRALTGIAVEQDKNTQEVFAQVKQIYKTPPIKDFGGFNFSQILPDPSKPSKRSFIEDLLFNKVTLADAGFIKQYGDCLGDIAARDLICAQKFNGLTVLPPLLTDEMIAQYTSALLAGTITSGWTFGAGAALQIPFAMQMAYRFNGIGVTQNVLYENQKLIANQFNSAIGKIQDSLSSTASALGKLQDVVNQNAQALNTLVKQLSSNFGAISSVLNDILSRLDKVEAEVQIDRLITGRLQSLQTYVTQQLIRAAEIRASANLAATKMSECVLGQSKRVDFCGKGYHLMSFPQSAPHGVVFLHVTYVPAQEKNFTTAPAICHDGKAHFPREGVFVSNGTHWFVTQRNFYEPQIITTDNTFVSGNCDVVIGIVNNTVYDPLQPELDSFKEELDKYFKNHTSPDVDLGDISGINASVVNIQKEIDRLNEVAKNLNESLIDLQELGKYEQYIKWPWYIWLGFIAGLIAIVMVTIMLCCMTSCCSCLKGCCSCGSCCKFDEDDSEPVLKGVKLHYT

SEQ ID NO: 10 - protein, 1273 aa, Artificial Sequence
  Artificial Sequence
MFVFLVLLPLVSSQCVNLTTRTQLPPAYTNSFTRGVYYPDKVFRSSVLHSTQDLFLPFFSNVTWFHAIHVSGTNGTKRFDNPVLPFNDGVYFASTEKSNIIRGWIFGTTLDSKTQSLLIVNNATNVVIKVCEFQFCNDPFLGVYYHKNNKSWMESEFRVYSSANNCTFEYVSQPFLMDLEGKQGNFKNLREFVFKNIDGYFKIYSKHTPINLVRDLPQGFSALEPLVDLPIGINITRFQTLLALHRSYLTPGDSSSGWTAGAAAYYVGYLQPRTFLLKYNENGTITDAVDCALDPLSETKCTLKSFTVEKGIYQTSNFRVQPTESIVRFPNITNLCPFGEVFNATRFASVYAWNRKRISNCVADYSVLYNSASFSTFKCYGVSPTKLNDLCFTNVYADSFVIRGDEVRQIAPGQTGKIADYNYKLPDDFTGCVIAWNSNNLDSKVGGNYNYLYRLFRKSNLKPFERDISTEIYQAGSTPCNGVEGFNCYFPLQSYGFQPTNGVGYQPYRVVVLSFELLHAPATVCGPKKSTNLVKNKCVNFNFNGLTGTGVLTESNKKFLPFQQFGRDIADTTDAVRDPQTLEILDITPCSFGGVSVITPGTNTSNQVAVLYQDVNCTEVPVAIHADQLTPTWRVYSTGSNVFQTRAGCLIGAEHVNNSYECDIPIGAGICASYQTQTNSPSRASSVASQSIIAYTMSLGAENSVAYSNNSIAIPTNFTISVTTEILPVSMTKTSVDCTMYICGDSTECSNLLLQYGSFCTQLNRALTGIAVEQDKNTQEVFAQVKQIYKTPPIKDFGGFNFSQILPDPSKPSKRSFIEDLLFNKVTLADAGFIKQYGDCLGDIAARDLICAQKFNGLTVLPPLLTDEMIAQYTSALLAGTITSGWTFGAGAALQIPFAMQMAYRFNGIGVTQNVLYENQKLIANQFNSAIGKIQDSLSSTASALGKLQDVVNQNAQALNTLVKQLSSNFGAISSVLNDILSRLDKVEAEVQIDRLITGRLQSLQTYVTQQLIRAAEIRASANLAATKMSECVLGQSKRVDFCGKGYHLMSFPQSAPHGVVFLHVTYVPAQEKNFTTAPAICHDGKAHFPREGVFVSNGTHWFVTQRNFYEPQIITTDNTFVSGNCDVVIGIVNNTVYDPLQPELDSFKEELDKYFKNHTSPDVDLGDISGINASVVNIQKEIDRLNEVAKNLNESLIDLQELGKYEQYIKWPWYIWLGFIAGLIAIVMVTIMLCCMTSCCSCLKGCCSCGSCCKFDEDDSEPVLKGVKLHYT

SEQ ID NO: 11 - protein, 1208 aa, Artificial Sequence
  Artificial Sequence
MFVFLVLLPLVSSQCVNLTTRTQLPPAYTNSFTRGVYYPDKVFRSSVLHSTQDLFLPFFSNVTWFHAIHVSGTNGTKRFDNPVLPFNDGVYFASTEKSNIIRGWIFGTTLDSKTQSLLIVNNATNVVIKVCEFQFCNDPFLGVYYHKNNKSWMESEFRVYSSANNCTFEYVSQPFLMDLEGKQGNFKNLREFVFKNIDGYFKIYSKHTPINLVRDLPQGFSALEPLVDLPIGINITRFQTLLALHRSYLTPGDSSSGWTAGAAAYYVGYLQPRTFLLKYNENGTITDAVDCALDPLSETKCTLKSFTVEKGIYQTSNFRVQPTESIVRFPNITNLCPFGEVFNATRFASVYAWNRKRISNCVADYSVLYNSASFSTFKCYGVSPTKLNDLCFTNVYADSFVIRGDEVRQIAPGQTGKIADYNYKLPDDFTGCVIAWNSNNLDSKVGGNYNYLYRLFRKSNLKPFERDISTEIYQAGSTPCNGVEGFNCYFPLQSYGFQPTNGVGYQPYRVVVLSFELLHAPATVCGPKKSTNLVKNKCVNFNFNGLTGTGVLTESNKKFLPFQQFGRDIADTTDAVRDPQTLEILDITPCSFGGVSVITPGTNTSNQVAVLYQDVNCTEVPVAIHADQLTPTWRVYSTGSNVFQTRAGCLIGAEHVNNSYECDIPIGAGICASYQTQTNSPRRARSVASQSIIAYTMSLGAENSVAYSNNSIAIPTNFTISVTTEILPVSMTKTSVDCTMYICGDSTECSNLLLQYGSFCTQLNRALTGIAVEQDKNTQEVFAQVKQIYKTPPIKDFGGFNFSQILPDPSKPSKRSFIEDLLFNKVTLADAGFIKQYGDCLGDIAARDLICAQKFNGLTVLPPLLTDEMIAQYTSALLAGTITSGWTFGAGAALQIPFAMQMAYRFNGIGVTQNVLYENQKLIANQFNSAIGKIQDSLSSTASALGKLQDVVNQNAQALNTLVKQLSSNFGAISSVLNDILSRLDKVEAEVQIDRLITGRLQSLQTYVTQQLIRAAEIRASANLAATKMSECVLGQSKRVDFCGKGYHLMSFPQSAPHGVVFLHVTYVPAQEKNFTTAPAICHDGKAHFPREGVFVSNGTHWFVTQRNFYEPQIITTDNTFVSGNCDVVIGIVNNTVYDPLQPELDSFKEELDKYFKNHTSPDVDLGDISGINASVVNIQKEIDRLNEVAKNLNESLIDLQELGKYEQ

SEQ ID NO: 12 - protein, 1208 aa, Artificial Sequence
  Artificial Sequence
MFVFLVLLPLVSSQCVNLTTRTQLPPAYTNSFTRGVYYPDKVFRSSVLHSTQDLFLPFFSNVTWFHAIHVSGTNGTKRFDNPVLPFNDGVYFASTEKSNIIRGWIFGTTLDSKTQSLLIVNNATNVVIKVCEFQFCNDPFLGVYYHKNNKSWMESEFRVYSSANNCTFEYVSQPFLMDLEGKQGNFKNLREFVFKNIDGYFKIYSKHTPINLVRDLPQGFSALEPLVDLPIGINITRFQTLLALHRSYLTPGDSSSGWTAGAAAYYVGYLQPRTFLLKYNENGTITDAVDCALDPLSETKCTLKSFTVEKGIYQTSNFRVQPTESIVRFPNITNLCPFGEVFNATRFASVYAWNRKRISNCVADYSVLYNSASFSTFKCYGVSPTKLNDLCFTNVYADSFVIRGDEVRQIAPGQTGKIADYNYKLPDDFTGCVIAWNSNNLDSKVGGNYNYLYRLFRKSNLKPFERDISTEIYQAGSTPCNGVEGFNCYFPLQSYGFQPTNGVGYQPYRVVVLSFELLHAPATVCGPKKSTNLVKNKCVNFNFNGLTGTGVLTESNKKFLPFQQFGRDIADTTDAVRDPQTLEILDITPCSFGGVSVITPGTNTSNQVAVLYQDVNCTEVPVAIHADQLTPTWRVYSTGSNVFQTRAGCLIGAEHVNNSYECDIPIGAGICASYQTQTNSPSRASSVASQSIIAYTMSLGAENSVAYSNNSIAIPTNFTISVTTEILPVSMTKTSVDCTMYICGDSTECSNLLLQYGSFCTQLNRALTGIAVEQDKNTQEVFAQVKQIYKTPPIKDFGGFNFSQILPDPSKPSKRSFIEDLLFNKVTLADAGFIKQYGDCLGDIAARDLICAQKFNGLTVLPPLLTDEMIAQYTSALLAGTITSGWTFGAGAALQIPFAMQMAYRFNGIGVTQNVLYENQKLIANQFNSAIGKIQDSLSSTASALGKLQDVVNQNAQALNTLVKQLSSNFGAISSVLNDILSRLDKVEAEVQIDRLITGRLQSLQTYVTQQLIRAAEIRASANLAATKMSECVLGQSKRVDFCGKGYHLMSFPQSAPHGVVFLHVTYVPAQEKNFTTAPAICHDGKAHFPREGVFVSNGTHWFVTQRNFYEPQIITTDNTFVSGNCDVVIGIVNNTVYDPLQPELDSFKEELDKYFKNHTSPDVDLGDISGINASVVNIQKEIDRLNEVAKNLNESLIDLQELGKYEQ

SEQ ID NO: 13 - protein, 1443 aa, Artificial Sequence
  Artificial
MPLLLLLPLLWAGALATIEEQAKTFLDKFNHEAEDLFYQSSLASWNYNTNITEENVQNMNNAGDKWSAFLKEQSTLAQMYPLQEIQNLTVKLQLQALQQNGSSVLSEDKSKRLNTILNTMSTIYSTGKVCNPDNPQECLLLEPGLNEIMANSLDYNERLWAWESWRSEVGKQLRPLYEEYVVLKNEMARANHYEDYGDYWRGDYEVNGVDGYDYSRGQLIEDVEHTFEEIKPLYEHLHAYVRAKLMNAYPSYISPIGCLPAHLLGDMWGRFWTNLYSLTVPFGQKPNIDVTDAMVDQAWDAQRIFKEAEKFFVSVGLPNMTQGFWENSMLTDPGNVQKAVCHPTAWDLGKGDFRILMCTKVTMDDFLTAHNEMGNIQYDMAYAAQPFLLRNGANEGFHEAVGEIMSLSAATPKHLKSIGLLSPDFQEDNETEINFLLKQALTIVGTLPFTYMLEKWRWMVFKGEIPKDQWMKKWWEMKREIVGVVEPVPHDETYCDPASLFHVSNDYSFIRYYTRTLYQFQFQEALCQAAKHEGPLHKCDISNSTEAGQKLFNMLRLGKSEPWTLALENVVGAKNMNVRPLLNYFEPLFTWLKDQNKNSFVGWSTDWSPYADEPKSSDKTHTCPPCPAPELLGGPSVFLFPPKPKDTLMISRTPEVTCVVVDVSHEDPEVKFNWYVDGVEVHNAKTKPREEQYNSTYRVVSVLTVLHQDWLNGKEYKCKVSNKALPAPIEKTISKAKGQPREPQVYTLPPSRDELTKNQVSLTCLVKGFYPSDIAVEWESNGQPENNYKTTPPVLDSDGSFFLYSKLTVDKSRWQQGNVFSCSVMHEALHNHYTQKSLSLSPGKAAATIEEQAKTFLDKFNHEAEDLFYQSSLASWNYNTNITEENVQNMNNAGDKWSAFLKEQSTLAQMYPLQEIQNLTVKLQLQALQQNGSSVLSEDKSKRLNTILNTMSTIYSTGKVCNPDNPQECLLLEPGLNEIMANSLDYNERLWAWESWRSEVGKQLRPLYEEYVVLKNEMARANHYEDYGDYWRGDYEVNGVDGYDYSRGQLIEDVEHTFEEIKPLYEHLHAYVRAKLMNAYPSYISPIGCLPAHLLGDMWGRFWTNLYSLTVPFGQKPNIDVTDAMVDQAWDAQRIFKEAEKFFVSVGLPNMTQGFWENSMLTDPGNVQKAVCHPTAWDLGKGDFRILMCTKVTMDDFLTAHNEMGNIQYDMAYAAQPFLLRNGANEGFHEAVGEIMSLSAATPKHLKSIGLLSPDFQEDNETEINFLLKQALTIVGTLPFTYMLEKWRWMVFKGEIPKDQWMKKWWEMKREIVGVVEPVPHDETYCDPASLFHVSNDYSFIRYYTRTLYQFQFQEALCQAAKHEGPLHKCDISNSTEAGQKLFNMLRLGKSEPWTLALENVVGAKNMNVRPLLNYFEPLFTWLKDQNKNSFVGWSTDWSPYAD

SEQ ID NO: 14 - protein, 1440 aa, Artificial Sequence
  Artificial
MPLLLLLPLLWAGALATIEEQAKTFLDKFNHEAEDLFYQSSLASWNYNTNITEENVQNMNNAGDKWSAFLKEQSTLAQMYPLQEIQNLTVKLQLQALQQNGSSVLSEDKSKRLNTILNTMSTIYSTGKVCNPDNPQECLLLEPGLNEIMANSLDYNERLWAWESWRSEVGKQLRPLYEEYVVLKNEMARANHYEDYGDYWRGDYEVNGVDGYDYSRGQLIEDVEHTFEEIKPLYEHLHAYVRAKLMNAYPSYISPIGCLPAHLLGDMWGRFWTNLYSLTVPFGQKPNIDVTDAMVDQAWDAQRIFKEAEKFFVSVGLPNMTQGFWENSMLTDPGNVQKAVCHPTAWDLGKGDFRILMCTKVTMDDFLTAHNEMGNIQYDMAYAAQPFLLRNGANEGFHEAVGEIMSLSAATPKHLKSIGLLSPDFQEDNETEINFLLKQALTIVGTLPFTYMLEKWRWMVFKGEIPKDQWMKKWWEMKREIVGVVEPVPHDETYCDPASLFHVSNDYSFIRYYTRTLYQFQFQEALCQAAKHEGPLHKCDISNSTEAGQKLFNMLRLGKSEPWTLALENVVGAKNMNVRPLLNYFEPLFTWLKDQNKNSFVGWSTDWSPYADTIEEQAKTFLDKFNHEAEDLFYQSSLASWNYNTNITEENVQNMNNAGDKWSAFLKEQSTLAQMYPLQEIQNLTVKLQLQALQQNGSSVLSEDKSKRLNTILNTMSTIYSTGKVCNPDNPQECLLLEPGLNEIMANSLDYNERLWAWESWRSEVGKQLRPLYEEYVVLKNEMARANHYEDYGDYWRGDYEVNGVDGYDYSRGQLIEDVEHTFEEIKPLYEHLHAYVRAKLMNAYPSYISPIGCLPAHLLGDMWGRFWTNLYSLTVPFGQKPNIDVTDAMVDQAWDAQRIFKEAEKFFVSVGLPNMTQGFWENSMLTDPGNVQKAVCHPTAWDLGKGDFRILMCTKVTMDDFLTAHNEMGNIQYDMAYAAQPFLLRNGANEGFHEAVGEIMSLSAATPKHLKSIGLLSPDFQEDNETEINFLLKQALTIVGTLPFTYMLEKWRWMVFKGEIPKDQWMKKWWEMKREIVGVVEPVPHDETYCDPASLFHVSNDYSFIRYYTRTLYQFQFQEALCQAAKHEGPLHKCDISNSTEAGQKLFNMLRLGKSEPWTLALENVVGAKNMNVRPLLNYFEPLFTWLKDQNKNSFVGWSTDWSPYADEPKSSDKTHTCPPCPAPELLGGPSVFLFPPKPKDTLMISRTPEVTCVVVDVSHEDPEVKFNWYVDGVEVHNAKTKPREEQYNSTYRVVSVLTVLHQDWLNGKEYKCKVSNKALPAPIEKTISKAKGQPREPQVYTLPPSRDELTKNQVSLTCLVKGFYPSDIAVEWESNGQPENNYKTTPPVLDSDGSFFLYSKLTVDKSRWQQGNVFSCSVMHEALHNHYTQKSLSLSPGK

SEQ ID NO: 15 - protein, 18 aa, Artificial Sequence
  Artificial
PTLYNVSLVMSDTAGTCY

SEQ ID NO: 16 - protein, 18 aa, Artificial Sequence
  Artificial
PTHVNVSVVMAEVDGTCY

SEQ ID NO: 17 - protein, 21 aa, Artificial Sequence
  Artificial
TGKPTLYNVSLVMSDTAGTCY

SEQ ID NO: 18 - protein, 862 aa, Artificial Sequence
  Artificial
MPLLLLLPLLWAGALATIEEQAKTFLDKFNHEAEDLFYQSSLASWNYNTNITEENVQNMNNAGDKWSAFLKEQSTLAQMYPLQEIQNLTVKLQLQALQQNGSSVLSEDKSKRLNTILNTMSTIYSTGKVCNPDNPQECLLLEPGLNEIMANSLDYNERLWAWESWRSEVGKQLRPLYEEYVVLKNEMARANHYEDYGDYWRGDYEVNGVDGYDYSRGQLIEDVEHTFEEIKPLYEHLHAYVRAKLMNAYPSYISPIGCLPAHLLGDMWGRFWTNLYSLTVPFGQKPNIDVTDAMVDQAWDAQRIFKEAEKFFVSVGLPNMTQGFWENSMLTDPGNVQKAVCHPTAWDLGKGDFRILMCTKVTMDDFLTAHNEMGNIQYDMAYAAQPFLLRNGANEGFHEAVGEIMSLSAATPKHLKSIGLLSPDFQEDNETEINFLLKQALTIVGTLPFTYMLEKWRWMVFKGEIPKDQWMKKWWEMKREIVGVVEPVPHDETYCDPASLFHVSNDYSFIRYYTRTLYQFQFQEALCQAAKHEGPLHKCDISNSTEAGQKLFNMLRLGKSEPWTLALENVVGAKNMNVRPLLNYFEPLFTWLKDQNKNSFVGWSTDWSPYADEPKSSDKTHTCPPCPAPELLGGPSVFLFPPKPKDTLMISRTPEVTCVVVDVSHEDPEVKFNWYVDGVEVHNAKTKPREEQYNSTYRVVSVLTVCHQDWLNGKEYKCKVSNKALPAPIEKTISKAKGQPREPQVYTLPPSRDELTKNQVSLTCLVKGFYPSDIAVEWESNGQPENNYKTTPPVLDSDGSFFLYSKLTVDKSRWQQGNVFSCSVMHEALHNHYTQKSLSLSTGKPTLYNVSLVMSDTAGTCY